European Patent Specification EP 4 061 366 B1, published February 25, 2026. Title: INHIBITORS OF HISTONE DEMETHYLASES. Applicant: THE UNITED STATES OF AMERICA, AS REPRESENTED BY THE SECRETARY, DEPARTMENT OF HEALTH AND HUMAN SERVICES. The sequence listing filed with the application follows.

SEQUENCE LISTING (1 sequence)

SEQ ID NO: 1 - DNA, 608 bp, Artificial Sequence
  synthetic
tgcctgggtaaagaagctagggaattgggggatatggacatagagtgatcatgtttattctctttccaacaaaggcctgaattaacaaacacaaaatggctctgctgctaagaaaaacacagtgggtagatacacttgaaagtcacttctgaaagagaccttgaagaagggatggagaatgtttggggtggacagaaactcctccaagaaagacaatgaaagacaacaagttaggtcacggtggctaaagaggagacaatgatttgttgtctgactctccagctacgatggggctgtaactaatgaggttattctggttacaaaggaagcattcagccccttaatgaaaaactctttggcaactggtgttagggaaagaaaaaacaaaccagcagcttattattagttccacagcaagttaattaatttttgccagtcactttgggtcacttgctggactgagcatctgtctcactcaactgaacagctggagggatggtgggtgtctctgcgggccatgcatgtgtcctgttccgggaggagaagggagagctaactacaaggctgaaaaaacgtgagcttccagtgttcatctgctcctctcctgt